European Patent Specification EP 3 735 476 B1, published August 23, 2023. Title: Method for determining the presence or absence of M. tuberculosis, M. bovis and M. bovis BCG in a Sample. Applicant: Seegene, INC. The sequence listing filed with the application follows.

SEQUENCE LISTING (36 sequences)

SEQ ID NO: 1 - DNA, 296 bp, Mycobacterium sp.
gggcaagacgaccattgcccacgcgatcgcgcgcgccatttgtgcccgaaacagtccccagcaggtgcggttcatgctcgcggactaccgctcgggcctgctggacgcggtgccggacacccatctgctgggcgccggcgcgatcaaccgcaacagcgcgtcgctagacgaggccgttcaagcactggcggtcaacctgaagaagcggttgccgccgaccgacctgacgacggcgcagctacgctcgcgttcgtggtggagcggatttgacgtcgtgcttctggtcgacgattggc

SEQ ID NO: 2 - DNA, 306 bp, Mycobacterium sp.
cggttacgctggttaattatgacgtccgttaccaccgagcgccccgtgcgacagcgcggccagcgcaagcgaggtgaccacccggctgatcgcccaagcggtgcatcatgcgcgcggattcaacgggttactgcgaataccggcgcggggtggatccagcggccgagccggcgtgaaatgccggaggccaaccggacggtgatccgcgaggcgatctggcggtttggggagggcagtaggggatgagtattaccaggccgacgggcagctatgccagacagatgctggatccgggcggctggatgt

SEQ ID NO: 3 - DNA, 306 bp, Mycobacterium sp.
acatccagccgcccggatccagcatctgtctggcatagctgcccgtcggcctggtaatactcatcccctactgccctccccaaaccgccagatcgcctcgcggatcaccgtccggttggcctccggcatttcacgccggctcggccgctggatccaccccgcgccggtattcgcagtaacccgttgaatccgcgcgcatgatgcaccgcttgggcgatcagccgggtggtcacctcgcttgcgctggccgcgctgtcgcacggggcgctcggtggtaacggacgtcataattaaccagcgtaaccg

SEQ ID NO: 4 - DNA, 296 bp, Mycobacterium sp.
gccaatcgtcgaccagaagcacgacgtcaaatccgctccaccacgaacgcgagcgtagctgcgccgtcgtcaggtcggtcggcggcaaccgcttcttcaggttgaccgccagtgcttgaacggcctcgtctagcgacgcgctgttgcggttgatcgcgccggcgcccagcagatgggtgtccggcaccgcgtccagcaggcccgagcggtagtccgcgagcatgaaccgcacctgctggggactgtttcgggcacaaatggcgcgcgcgatcgcgtgggcaatggtcgtcttgccc

SEQ ID NO: 5 - DNA, 300 bp, Mycobacterium sp.
ccgttcagtttggcgtaggccagcgccacgaacatcgcgtgggactccggcggaaagcgttgtgcgacctcgtcgaaggccactaaaggcaggccgcaaaactcggacacgcttgcatagtctcggtcgactgtgaacgcgacgacctcatattccgaatcccttgtgaagtagtaatgtgcgagctgagcgatgtcgccgctcccaaaaattaccaatggtttggtcatgacgccttcctaaccagaattgtgaattcatacaagccgtagtcgtgcagaagcgcaacactcttggagt

SEQ ID NO: 6 - DNA, 300 bp, Mycobacterium sp.
catcgcgcatgaacaccagcacggctagcgcgatgccgacacccgccaccatgccgcccacccagaaggcgaacagattcagcatgggccgacgccgcgacagcatgacgaccgcgagtcccagacgcgccgggtcaatcgccatccccaaccccaaaaggagcaccatcgtccacatcagtggggacgctactacggcacggcgcgccccgtagcgttactgagaaattgctgaaaaatggctattgaccagctaagatatccggtacgcccgcgccgcggagagcgccgttgtaggcc

SEQ ID NO: 7 - DNA, 300 bp, Mycobacterium sp.
ggcctacaacggcgctctccgcggcgcgggcgtaccggatatcttagctggtcaatagccatttttcagcaatttctcagtaacgctacggggcgcgccgtgccgtagtagcgtccccactgatgtggacgatggtgctccttttggggttggggatggcgattgacccggcgcgtctgggactcgcggtcgtcatgctgtcgcggcgtcggcccatgctgaatctgttcgccttctgggtgggcggcatggtggcgggtgtcggcatcgcgctagccgtgctggtgttcatgcgcgatg

SEQ ID NO: 8 - DNA, 300 bp, Mycobacterium sp.
actccaagagtgttgcgcttctgcacgactacggcttgtatgaattcacaattctggttaggaaggcgtcatgaccaaaccattggtaatttttgggagcggcgacatcgctcagctcgcacattactacttcacaagggattcggaatatgaggtcgtcgcgttcacagtcgaccgagactatgcaagcgtgtccgagttttgcggcctgcctttagtggccttcgacgaggtcgcacaacgctttccgccggagtcccacgcgatgttcgtggcgctggcctacgccaaactgaacgg

SEQ ID NO: 9 - DNA, 58 bp, Mycobacterium sp.
ggtcccaatcgaaggccttgtacgtggtcgttgggtgcgtgccgccggcgttctggta

SEQ ID NO: 10 - DNA, 60 bp, Mycobacterium sp.
gattttcttcttcaacccgggggagttgctgcccgaagcagccggcccaacccaggtatt

SEQ ID NO: 11 - DNA, 61 bp, Mycobacterium sp.
cagccgtggacgacacgggcgctgctccggtagtaattttcggcggccgcagccagatcgg

SEQ ID NO: 12 - DNA, 58 bp, Mycobacterium sp.
ctggcgtttctttccgaacgccatctggccatgctgaccacgctgcgggcggacaact

SEQ ID NO: 13 - DNA, 58 bp, Mycobacterium sp.
ccgtcgtcaggtcggtcggcggcaaccgcttcttcaggttgaccgccagtgcttgaac

SEQ ID NO: 14 - DNA, 58 bp, Mycobacterium sp.
gcaccgcttgggcgatcagccgggtggtcacctcgcttgcgctggccgcgctgtcgca

SEQ ID NO: 15 - DNA, 58 bp, Mycobacterium sp.
tcacaagggattcggaatatgaggtcgtcgcgttcacagtcgaccgagactatgcaag

SEQ ID NO: 16 - DNA, 63 bp, Mycobacterium sp.
gctggtcaatagccatttttcagcaatttctcagtaacgctacggggcgcgccgtgccgtagt

SEQ ID NO: 17 - DNA, 65 bp, Mycobacterium sp.
aaggtgaactgagcaagcagaccggacaacaggtatcgatagcgccgaatgccggcttggacccg

SEQ ID NO: 18 - DNA, 62 bp, Mycobacterium sp.
agatggcgttcggaaagaaacgccagcgcgtcgtcactaagccgcgtagtggtgttgaccat

SEQ ID NO: 19 - DNA, 62 bp, Mycobacterium sp.
agacagatgctggatccgggcggctggatgtgccaatcgtcgaccagaagcacgacgtcaaa

SEQ ID NO: 20 - DNA, 64 bp, Mycobacterium sp.
tgtgcgagctgagcgatgtcgccgctcccaaaaattaccaatggtttggtcatgacgccttcct

SEQ ID NO: 21 - DNA, 18 bp, Artificial Sequence
  MPB64 F Primer
gcacccaacgaccacgta

SEQ ID NO: 22 - DNA, 18 bp, Artificial Sequence
  MPB64 R Primer
cttcgggcagcaactccc

SEQ ID NO: 23 - DNA, 25 bp, Artificial Sequence
  MPB64 Probe
gcgctatcgatacctgttgtccggt

SEQ ID NO: 24 - DNA, 21 bp, Artificial Sequence
  RD9 F Primer
gaaaattactaccggagcagc

SEQ ID NO: 25 - DNA, 18 bp, Artificial Sequence
  RD9 R Primer
gtcagcatggccagatgg

SEQ ID NO: 26 - DNA, 22 bp, Artificial Sequence
  RD9 Probe
gcttagtgacgacgcgctggcg

SEQ ID NO: 27 - DNA, 18 bp, Artificial Sequence
  RD1del F Primer
cctgaagaagcggttgcc

SEQ ID NO: 28 - DNA, 18 bp, Artificial Sequence
  RD1del R Primer
aagcgaggtgaccacccg

SEQ ID NO: 29 - DNA, 22 bp, Artificial Sequence
  RD1del Probe
cgacgattggcacatccagccg

SEQ ID NO: 30 - DNA, 18 bp, Artificial Sequence
  RD4del F Primer
tgtgaacgcgacgacctc

SEQ ID NO: 31 - DNA, 23 bp, Artificial Sequence
  RD4del R Primer
gtagcgttactgagaaattgctg

SEQ ID NO: 32 - DNA, 24 bp, Artificial Sequence
  RD4del Probe
ccattggtaatttttgggagcggc

SEQ ID NO: 33 - DNA, 702 bp, Mycobacterium sp.
acaacatcaacatcagcctgcccagttactaccccgaccagaagtcgctggaaaattacatcgcccagacgcgcgacaagttcctcagcgcggccacatcgtccactccacgcgaagccccctacgaattgaatatcacctcggccacataccagtccgcgataccgccgcgtggtacgcaggccgtggtgctcaaggtctaccagaacgccggcggcacgcacccaacgaccacgtacaaggccttcgattgggaccaggcctatcgcaagccaatcacctatgacacgctgtggcaggctgacaccgatccgctgccagtcgtcttccccattgtgcaaggtgaactgagcaagcagaccggacaacaggtatcgatagcgccgaatgccggcttggacccggtgaattatcagaacttcgcagtcacgaacgacggggtgattttcttcttcaacccgggggagttgctgcccgaagcagccggcccaacccaggtattggtcccacgttccgcgatcgactcgatgctggcctagactcgcgaggaccgcgcggtggtcactgcgcggatttggggcggcggaagtgagtgttcggtgcgcccactgcggtgactcacctgcagcgccggcatcgacaggccgggagctcaagaatcgtcgctagagaatctatggtgcgttagaggattccctgcta

SEQ ID NO: 34 - DNA, 702 bp, Mycobacterium sp.
tagcagggaatcctctaacgcaccatagattctctagcgacgattcttgagctcccggcctgtcgatgccggcgctgcaggtgagtcaccgcagtgggcgcaccgaacactcacttccgccgccccaaatccgcgcagtgaccaccgcgcggtcctcgcgagtctaggccagcatcgagtcgatcgcggaacgtgggaccaatacctgggttgggccggctgcttcgggcagcaactcccccgggttgaagaagaaaatcaccccgtcgttcgtgactgcgaagttctgataattcaccgggtccaagccggcattcggcgctatcgatacctgttgtccggtctgcttgctcagttcaccttgcacaatggggaagacgactggcagcggatcggtgtcagcctgccacagcgtgtcataggtgattggcttgcgataggcctggtcccaatcgaaggccttgtacgtggtcgttgggtgcgtgccgccggcgttctggtagaccttgagcaccacggcctgcgtaccacgcggcggtatcgcggactggtatgtggccgaggtgatattcaattcgtagggggcttcgcgtggagtggacgatgtggccgcgctgaggaacttgtcgcgcgtctgggcgatgtaattttccagcgacttctggtcggggtagtaactgggcaggctgatgttgatgttgt

SEQ ID NO: 35 - DNA, 585 bp, Mycobacterium sp.
ggcgtcgcgcacggcgtcgatgtcgctgttcaccgccgccctaccctccagtgagagccagcgcgcgccgtcgacctggctgagcacggcaagcccactgcggtcggcattgacggccttttgggagccgccggtggtgatgacccgcgcgatgtgagtcttggggtcgaaggtgaaacctaccgccaccacgtgcggcgagttgtccgcccgcagcgtggtcagcatggccagatggcgttcggaaagaaacgccagcgcgtcgtcactaagccgcgtagtggtgttgaccatcgccactcacgctagcgcaggcaataatcgcagccgtggacgacacgggcgctgctccggtagtaattttcggcggccgcagccagatcggcggcgaactcgcgcgacgcctggctgccggggcgacgatggtgctggccgcgcggaacgccgatcaactcgccgaccaggccgccgcactccgcgcagctggcgctatagcggtgcacacccgggagttcgacgccgacgacctggccgcacacggcccgttggtcgcttcgctcgttgccgagcacggccccatcggca

SEQ ID NO: 36 - DNA, 585 bp, Mycobacterium sp.
tgccgatggggccgtgctcggcaacgagcgaagcgaccaacgggccgtgtgcggccaggtcgtcggcgtcgaactcccgggtgtgcaccgctatagcgccagctgcgcggagtgcggcggcctggtcggcgagttgatcggcgttccgcgcggccagcaccatcgtcgccccggcagccaggcgtcgcgcgagttcgccgccgatctggctgcggccgccgaaaattactaccggagcagcgcccgtgtcgtccacggctgcgattattgcctgcgctagcgtgagtggcgatggtcaacaccactacgcggcttagtgacgacgcgctggcgtttctttccgaacgccatctggccatgctgaccacgctgcgggcggacaactcgccgcacgtggtggcggtaggtttcaccttcgaccccaagactcacatcgcgcgggtcatcaccaccggcggctcccaaaaggccgtcaatgccgaccgcagtgggcttgccgtgctcagccaggtcgacggcgcgcgctggctctcactggagggtagggcggcggtgaacagcgacatcgacgccgtgcgcgacgcc